European Patent Application EP 4 491 189 A1, published January 15, 2025. Title: COMPOSITION FOR PREVENTING OR TREATING DENTAL CARIES. Applicant: HYSENSBIO CO., LTD. Application KR. The sequence listing filed with the application follows.

SEQUENCE LISTING (106 sequences)

SEQ ID NO: 1 - protein, 10 aa, synthetic construct
  REGION 1..10: note = Novel peptide
KYQRRKKNKY

SEQ ID NO: 2 - protein, 10 aa, synthetic construct
  REGION 1..10: note = Novel peptide
KYQRRKRNKY

SEQ ID NO: 3 - protein, 10 aa, synthetic construct
  REGION 1..10: note = Novel peptide
KYQRRRKNKY

SEQ ID NO: 4 - protein, 10 aa, synthetic construct
  REGION 1..10: note = Novel peptide
KYQRRRRNKY

SEQ ID NO: 5 - protein, 10 aa, synthetic construct
  REGION 1..10: note = Novel peptide
KYQRKKKNKY

SEQ ID NO: 6 - protein, 10 aa, synthetic construct
  REGION 1..10: note = Novel peptide
KYQRKRKNKY

SEQ ID NO: 7 - protein, 10 aa, synthetic construct
  REGION 1..10: note = Novel peptide
KYQRKKRNKY

SEQ ID NO: 8 - protein, 10 aa, synthetic construct
  REGION 1..10: note = Novel peptide
KYQRKRRNKY

SEQ ID NO: 9 - protein, 10 aa, synthetic construct
  REGION 1..10: note = Novel peptide
KYQRRKKSKY

SEQ ID NO: 10 - protein, 10 aa, synthetic construct
  REGION 1..10: note = Novel peptide
KYQRRKRSKY

SEQ ID NO: 11 - protein, 10 aa, synthetic construct
  REGION 1..10: note = Novel peptide
KYQRRRKSKY

SEQ ID NO: 12 - protein, 10 aa, synthetic construct
  REGION 1..10: note = Novel peptide
KYQRRRRSKY

SEQ ID NO: 13 - protein, 10 aa, synthetic construct
  REGION 1..10: note = Novel peptide
KYQRKKKSKY

SEQ ID NO: 14 - protein, 10 aa, synthetic construct
  REGION 1..10: note = Novel peptide
KYQRKRKSKY

SEQ ID NO: 15 - protein, 10 aa, synthetic construct
  REGION 1..10: note = Novel peptide
KYQRKKRSKY

SEQ ID NO: 16 - protein, 10 aa, synthetic construct
  REGION 1..10: note = Novel peptide
KYQRKRRSKY

SEQ ID NO: 17 - protein, 10 aa, synthetic construct
  REGION 1..10: note = Novel peptide
KYQRRKKNYK

SEQ ID NO: 18 - protein, 10 aa, synthetic construct
  REGION 1..10: note = Novel peptide
KYQRRKRNYK

SEQ ID NO: 19 - protein, 10 aa, synthetic construct
  REGION 1..10: note = Novel peptide
KYQRRRKNYK

SEQ ID NO: 20 - protein, 10 aa, synthetic construct
  REGION 1..10: note = Novel peptide
KYQRRRRNYK

SEQ ID NO: 21 - protein, 10 aa, synthetic construct
  REGION 1..10: note = Novel peptide
KYQRKKKNYK

SEQ ID NO: 22 - protein, 10 aa, synthetic construct
  REGION 1..10: note = Novel peptide
KYQRKRKNYK

SEQ ID NO: 23 - protein, 10 aa, synthetic construct
  REGION 1..10: note = Novel peptide
KYQRKKRNYK

SEQ ID NO: 24 - protein, 10 aa, synthetic construct
  REGION 1..10: note = Novel peptide
KYQRKRRNYK

SEQ ID NO: 25 - protein, 10 aa, synthetic construct
  REGION 1..10: note = Novel peptide
KYQRRKKSYK

SEQ ID NO: 26 - protein, 10 aa, synthetic construct
  REGION 1..10: note = Novel peptide
KYQRRKRSYK

SEQ ID NO: 27 - protein, 10 aa, synthetic construct
  REGION 1..10: note = Novel peptide
KYQRRRKSYK

SEQ ID NO: 28 - protein, 10 aa, synthetic construct
  REGION 1..10: note = Novel peptide
KYQRRRRSYK

SEQ ID NO: 29 - protein, 10 aa, synthetic construct
  REGION 1..10: note = Novel peptide
KYQRKKKSYK

SEQ ID NO: 30 - protein, 10 aa, synthetic construct
  REGION 1..10: note = Novel peptide
KYQRKRKSYK

SEQ ID NO: 31 - protein, 10 aa, synthetic construct
  REGION 1..10: note = Novel peptide
KYQRKKRSYK

SEQ ID NO: 32 - protein, 10 aa, synthetic construct
  REGION 1..10: note = Novel peptide
KYQRKRRSYK

SEQ ID NO: 33 - protein, 10 aa, synthetic construct
  REGION 1..10: note = Novel peptide
KYRQRKKNKY

SEQ ID NO: 34 - protein, 10 aa, synthetic construct
  REGION 1..10: note = Novel peptide
KYRQRKRNKY

SEQ ID NO: 35 - protein, 10 aa, synthetic construct
  REGION 1..10: note = Novel peptide
KYRQRRKNKY

SEQ ID NO: 36 - protein, 10 aa, synthetic construct
  REGION 1..10: note = Novel peptide
KYRQRRRNKY

SEQ ID NO: 37 - protein, 10 aa, synthetic construct
  REGION 1..10: note = Novel peptide
KYRQKKKNKY

SEQ ID NO: 38 - protein, 10 aa, synthetic construct
  REGION 1..10: note = Novel peptide
KYRQKRKNKY

SEQ ID NO: 39 - protein, 10 aa, synthetic construct
  REGION 1..10: note = Novel peptide
KYRQKKRNKY

SEQ ID NO: 40 - protein, 10 aa, synthetic construct
  REGION 1..10: note = Novel peptide
KYRQKRRNKY

SEQ ID NO: 41 - protein, 10 aa, synthetic construct
  REGION 1..10: note = Novel peptide
KYRQRKKSKY

SEQ ID NO: 42 - protein, 10 aa, synthetic construct
  REGION 1..10: note = Novel peptide
KYRQRKRSKY

SEQ ID NO: 43 - protein, 10 aa, synthetic construct
  REGION 1..10: note = Novel peptide
KYRQRRKSKY

SEQ ID NO: 44 - protein, 10 aa, synthetic construct
  REGION 1..10: note = Novel peptide
KYRQRRRSKY

SEQ ID NO: 45 - protein, 10 aa, synthetic construct
  REGION 1..10: note = Novel peptide
KYRQKKKSKY

SEQ ID NO: 46 - protein, 10 aa, synthetic construct
  REGION 1..10: note = Novel peptide
KYRQKRKSKY

SEQ ID NO: 47 - protein, 10 aa, synthetic construct
  REGION 1..10: note = Novel peptide
KYRQKKRSKY

SEQ ID NO: 48 - protein, 10 aa, synthetic construct
  REGION 1..10: note = Novel peptide
KYRQKRRSKY

SEQ ID NO: 49 - protein, 10 aa, synthetic construct
  REGION 1..10: note = Novel peptide
KYRQRKKNYK

SEQ ID NO: 50 - protein, 10 aa, synthetic construct
  REGION 1..10: note = Novel peptide
KYRQRKRNYK

SEQ ID NO: 51 - protein, 10 aa, synthetic construct
  REGION 1..10: note = Novel peptide
KYRQRRKNYK

SEQ ID NO: 52 - protein, 10 aa, synthetic construct
  REGION 1..10: note = Novel peptide
KYRQRRRNYK

SEQ ID NO: 53 - protein, 10 aa, synthetic construct
  REGION 1..10: note = Novel peptide
KYRQKKKNYK

SEQ ID NO: 54 - protein, 10 aa, synthetic construct
  REGION 1..10: note = Novel peptide
KYRQKRKNYK

SEQ ID NO: 55 - protein, 10 aa, synthetic construct
  REGION 1..10: note = Novel peptide
KYRQKKRNYK

SEQ ID NO: 56 - protein, 10 aa, synthetic construct
  REGION 1..10: note = Novel peptide
KYRQKRRNYK

SEQ ID NO: 57 - protein, 10 aa, synthetic construct
  REGION 1..10: note = Novel peptide
KYRQRKKSYK

SEQ ID NO: 58 - protein, 10 aa, synthetic construct
  REGION 1..10: note = Novel peptide
KYRQRKRSYK

SEQ ID NO: 59 - protein, 10 aa, synthetic construct
  REGION 1..10: note = Novel peptide
KYRQRRKSYK

SEQ ID NO: 60 - protein, 10 aa, synthetic construct
  REGION 1..10: note = Novel peptide
KYRQRRRSYK

SEQ ID NO: 61 - protein, 10 aa, synthetic construct
  REGION 1..10: note = Novel peptide
KYRQKKKSYK

SEQ ID NO: 62 - protein, 10 aa, synthetic construct
  REGION 1..10: note = Novel peptide
KYRQKRKSYK

SEQ ID NO: 63 - protein, 10 aa, synthetic construct
  REGION 1..10: note = Novel peptide
KYRQKKRSYK

SEQ ID NO: 64 - protein, 10 aa, synthetic construct
  REGION 1..10: note = Novel peptide
KYRQKRRSYK

SEQ ID NO: 65 - protein, 10 aa, synthetic construct
  REGION 1..10: note = Novel peptide
KYKQRKKNKY

SEQ ID NO: 66 - protein, 10 aa, synthetic construct
  REGION 1..10: note = Novel peptide
KYKQRKRNKY

SEQ ID NO: 67 - protein, 10 aa, synthetic construct
  REGION 1..10: note = Novel peptide
KYKQRRKNKY

SEQ ID NO: 68 - protein, 10 aa, synthetic construct
  REGION 1..10: note = Novel peptide
KYKQRRRNKY

SEQ ID NO: 69 - protein, 10 aa, synthetic construct
  REGION 1..10: note = Novel peptide
KYKQKKKNKY

SEQ ID NO: 70 - protein, 10 aa, synthetic construct
  REGION 1..10: note = Novel peptide
KYKQKRKNKY

SEQ ID NO: 71 - protein, 10 aa, synthetic construct
  REGION 1..10: note = Novel peptide
KYKQKKRNKY

SEQ ID NO: 72 - protein, 10 aa, synthetic construct
  REGION 1..10: note = Novel peptide
KYKQKRRNKY

SEQ ID NO: 73 - protein, 10 aa, synthetic construct
  REGION 1..10: note = Novel peptide
KYKQRKKSKY

SEQ ID NO: 74 - protein, 10 aa, synthetic construct
  REGION 1..10: note = Novel peptide
KYKQRKRSKY

SEQ ID NO: 75 - protein, 10 aa, synthetic construct
  REGION 1..10: note = Novel peptide
KYKQRRKSKY

SEQ ID NO: 76 - protein, 10 aa, synthetic construct
  REGION 1..10: note = Novel peptide
KYKQRRRSKY

SEQ ID NO: 77 - protein, 10 aa, synthetic construct
  REGION 1..10: note = Novel peptide
KYKQKKKSKY

SEQ ID NO: 78 - protein, 10 aa, synthetic construct
  REGION 1..10: note = Novel peptide
KYKQKRKSKY

SEQ ID NO: 79 - protein, 10 aa, synthetic construct
  REGION 1..10: note = Novel peptide
KYKQKKRSKY

SEQ ID NO: 80 - protein, 10 aa, synthetic construct
  REGION 1..10: note = Novel peptide
KYKQKRRSKY

SEQ ID NO: 81 - protein, 10 aa, synthetic construct
  REGION 1..10: note = Novel peptide
KYKQRKKNYK

SEQ ID NO: 82 - protein, 10 aa, synthetic construct
  REGION 1..10: note = Novel peptide
KYKQRKRNYK

SEQ ID NO: 83 - protein, 10 aa, synthetic construct
  REGION 1..10: note = Novel peptide
KYKQRRKNYK

SEQ ID NO: 84 - protein, 10 aa, synthetic construct
  REGION 1..10: note = Novel peptide
KYKQRRRNYK

SEQ ID NO: 85 - protein, 10 aa, synthetic construct
  REGION 1..10: note = Novel peptide
KYKQKKKNYK

SEQ ID NO: 86 - protein, 10 aa, synthetic construct
  REGION 1..10: note = Novel peptide
KYKQKRKNYK

SEQ ID NO: 87 - protein, 10 aa, synthetic construct
  REGION 1..10: note = Novel peptide
KYKQKKRNYK

SEQ ID NO: 88 - protein, 10 aa, synthetic construct
  REGION 1..10: note = Novel peptide
KYKQKRRNYK

SEQ ID NO: 89 - protein, 10 aa, synthetic construct
  REGION 1..10: note = Novel peptide
KYKQRKKSYK

SEQ ID NO: 90 - protein, 10 aa, synthetic construct
  REGION 1..10: note = Novel peptide
KYKQRKRSYK

SEQ ID NO: 91 - protein, 10 aa, synthetic construct
  REGION 1..10: note = Novel peptide
KYKQRRKSYK

SEQ ID NO: 92 - protein, 10 aa, synthetic construct
  REGION 1..10: note = Novel peptide
KYKQRRRSYK

SEQ ID NO: 93 - protein, 10 aa, synthetic construct
  REGION 1..10: note = Novel peptide
KYKQKKKSYK

SEQ ID NO: 94 - protein, 10 aa, synthetic construct
  REGION 1..10: note = Novel peptide
KYKQKRKSYK

SEQ ID NO: 95 - protein, 10 aa, synthetic construct
  REGION 1..10: note = Novel peptide
KYKQKKRSYK

SEQ ID NO: 96 - protein, 10 aa, synthetic construct
  REGION 1..10: note = Novel peptide
KYKQKRRSYK

SEQ ID NO: 97 - DNA, 20 bp, synthetic construct
  misc_feature 1..20: note = primer
  source 1..20: mol_type = other DNA
cgggacccattgaccaagtc

SEQ ID NO: 98 - DNA, 23 bp, synthetic construct
  misc_feature 1..23: note = primer
  source 1..23: mol_type = other DNA
catacacctcaaaccgtagcttc

SEQ ID NO: 99 - DNA, 23 bp, synthetic construct
  misc_feature 1..23: note = primer
  source 1..23: mol_type = other DNA
cctggtatgagcccatctatctg

SEQ ID NO: 100 - DNA, 23 bp, synthetic construct
  misc_feature 1..23: note = primer
  source 1..23: mol_type = other DNA
gcaatgatcccaaagtagacctg

SEQ ID NO: 101 - DNA, 24 bp, synthetic construct
  misc_feature 1..24: note = primer
  source 1..24: mol_type = other DNA
tgtatgtgactgcccaagatgaag

SEQ ID NO: 102 - DNA, 22 bp, synthetic construct
  misc_feature 1..22: note = primer
  source 1..22: mol_type = other DNA
agaggaggttggtctcactacc

SEQ ID NO: 103 - DNA, 21 bp, synthetic construct
  misc_feature 1..21: note = primer
  source 1..21: mol_type = other DNA
ccagggacaggatatggagca

SEQ ID NO: 104 - DNA, 23 bp, synthetic construct
  misc_feature 1..23: note = primer
  source 1..23: mol_type = other DNA
ttcaacacgcaggacaggtacag

SEQ ID NO: 105 - DNA, 21 bp, synthetic construct
  misc_feature 1..21: note = Aritificial Sequence
  source 1..21: mol_type = other DNA
cgaaagtcaactccatctgcc

SEQ ID NO: 106 - DNA, 21 bp, synthetic construct
  misc_feature 1..21: note = Aritificial Sequence
  source 1..21: mol_type = other DNA
ggcaactggctggaagtctct